European Patent Application EP 4 364 749 A1, published May 8, 2024. Title: PEPTIDES HAVING ANTI-OBESITY AND MUSCLE LOSS INHIBITORY ACTIVITY AND USES THEREOF. Applicant: Korea University Research and Business Foundation. The sequence listing filed with the application follows.

SEQUENCE LISTING (14 sequences)

SEQ ID NO: 1 - protein, 3 aa, Homo sapiens
YFR

SEQ ID NO: 2 - protein, 7 aa, Homo sapiens
EQAEEER

SEQ ID NO: 3 - protein, 10 aa, Homo sapiens
REAGGAFGKR

SEQ ID NO: 4 - protein, 10 aa, Homo sapiens
EQAEEERYFR

SEQ ID NO: 5 - protein, 12 aa, Homo sapiens
AQSREQLAALKK

SEQ ID NO: 6 - protein, 17 aa, Homo sapiens
YFRAQSREQLAALKKHH

SEQ ID NO: 7 - protein, 24 aa, Homo sapiens
AGSIREAGGAFGKREQAEEERYFR

SEQ ID NO: 8 - protein, 28 aa, Homo sapiens
VDRGAGSIREAGGAFGKREQAEEERYFR

SEQ ID NO: 9 - protein, 7 aa, Mus musculus
EKAEEDR

SEQ ID NO: 10 - protein, 10 aa, Mus musculus
EKAEEDRYFR

SEQ ID NO: 11 - protein, 14 aa, Mus musculus
EKTKEQLAALRKHH

SEQ ID NO: 12 - protein, 17 aa, Mus musculus
YFREKTKEQLAALRKHH

SEQ ID NO: 13 - protein, 24 aa, Mus musculus
AGSIREAGGAFGKREKAEEDRYFR

SEQ ID NO: 14 - protein, 28 aa, Mus musculus
MDTGAGSIREAGGAFGKREKAEEDRYFR